European Patent Specification EP 3 684 785 B1, published October 2, 2024. Title: N-METHYLATED CYCLIC PEPTIDES AND THEIR PRODRUGS. Applicant: Yissum Research Development Company of the Hebrew University of Jerusalem Ltd. TECHNISCHE UNIVERSITAT MUNCHEN. The sequence listing filed with the application follows.

SEQUENCE LISTING (24 sequences)

SEQ ID NO: 1 - protein, 6 aa, Artificial Sequence
  Cyclic peptide
  MISC_FEATURE (1)..(1): D-amino acid
  MISC_FEATURE (1)..(1): N-methylated
  MISC_FEATURE (5)..(5): N-methylated
RGDAAA

SEQ ID NO: 2 - protein, 6 aa, Artificial Sequence
  cyclic peptide
  MISC_FEATURE (1)..(1): D-amino acid
  MISC_FEATURE (1)..(1): N methylated
  MISC_FEATURE (6)..(6): N methylated
ARGDAA

SEQ ID NO: 3 - protein, 6 aa, Artificial Sequence
  Cyclic peptide
  MISC_FEATURE (1)..(1): D-amino acid
  MISC_FEATURE (3)..(3): N methylated
  MISC_FEATURE (5)..(5): N methylated
RGDAAA

SEQ ID NO: 4 - protein, 6 aa, Artificial Sequence
  Cyclic peptide
  MISC_FEATURE (1)..(1): D-amino acid
  MISC_FEATURE (5)..(5): N methylated
  MISC_FEATURE (6)..(6): N methylated
RGDAAA

SEQ ID NO: 5 - protein, 6 aa, Artificial Sequence
  Cyclic peptide
  MISC_FEATURE (1)..(1): D-amino acid
  MISC_FEATURE (1)..(1): N methylated
  MISC_FEATURE (6)..(6): N methylated
VRGDAA

SEQ ID NO: 6 - protein, 6 aa, Artificial Sequence
  Cyclic peptide
  MISC_FEATURE (1)..(1): D-amino acid
  MISC_FEATURE (1)..(1): N methylated
  MISC_FEATURE (6)..(6): N methylated
FRGDAA

SEQ ID NO: 7 - protein, 6 aa, Artificial Sequence
  Cyclic peptide
  MISC_FEATURE (1)..(1): D-amino acid
  MISC_FEATURE (1)..(1): N methylated
  MISC_FEATURE (5)..(5): N methylated
RGDAAV

SEQ ID NO: 8 - protein, 6 aa, Artificial Sequence
  Cyclic peptide
  MISC_FEATURE (1)..(1): D-amino acid
  MISC_FEATURE (1)..(1): N methylated
  MISC_FEATURE (5)..(5): N methylated
RGDAAF

SEQ ID NO: 9 - protein, 6 aa, Artificial Sequence
  Cyclic peptide
  MISC_FEATURE (1)..(1): D-amino acid
  MISC_FEATURE (1)..(1): N methylated
  MISC_FEATURE (2)..(2): Two hexyloxycarbonyl (Hoc) moieties
  MISC_FEATURE (4)..(4): Methyl ester (OMe) moiety
  MISC_FEATURE (6)..(6): N methylated
VRGDAA

SEQ ID NO: 10 - protein, 6 aa, Artificial Sequence
  Cyclic peptide
  MISC_FEATURE (1)..(1): D-amino acid
  MISC_FEATURE (1)..(1): N methylated
  MISC_FEATURE (2)..(2): Two hexyloxycarbonyl (Hoc) moieties
  MISC_FEATURE (4)..(4): Methyl ester (OMe) moiety
  MISC_FEATURE (6)..(6): N methylated
ARGDAA

SEQ ID NO: 11 - protein, 6 aa, Artificial Sequence
  Cyclic peptide
  MISC_FEATURE (1)..(1): D-amino acid
  MISC_FEATURE (1)..(1): N methylated
  MISC_FEATURE (1)..(1): Two hexyloxycarbonyl (Hoc) moieties
  MISC_FEATURE (3)..(3): Methyl ester (OMe) moiety
  MISC_FEATURE (5)..(5): N methylated
RGDAAA

SEQ ID NO: 12 - protein, 6 aa, Artificial Sequence
  Cyclic peptide
  MISC_FEATURE (1)..(1): D-amino acid
  MISC_FEATURE (1)..(1): Two hexyloxycarbonyl (Hoc) moieties
  MISC_FEATURE (3)..(3): Methyl ester (OMe) moiety
  MISC_FEATURE (5)..(5): N methylated
  MISC_FEATURE (6)..(6): N methylated
RGDAAA

SEQ ID NO: 13 - protein, 6 aa, Artificial Sequence
  Cyclic peptide
  MISC_FEATURE (1)..(1): D-amino acid
  MISC_FEATURE (1)..(1): Two hexyloxycarbonyl (Hoc) moieties
  MISC_FEATURE (3)..(3): N methylated
  MISC_FEATURE (3)..(3): Methyl ester (OMe) moiety
  MISC_FEATURE (5)..(5): N metylated
RGDAAA

SEQ ID NO: 14 - protein, 6 aa, Artificial Sequence
  Cyclic peptide
  MISC_FEATURE (1)..(1): D-amino acid
  MISC_FEATURE (1)..(1): N methylated
  MISC_FEATURE (2)..(2): Two hexyloxycarbonyl (Hoc) moieties
  MISC_FEATURE (4)..(4): Methyl ester (OMe) moiety
  MISC_FEATURE (6)..(6): N methylated
FRGDAA

SEQ ID NO: 15 - protein, 9 aa, Artificial Sequence
  Cyclic peptide
  MISC_FEATURE (5)..(5): Two hexyloxycarbonyl (Hoc) moieties
LPPFRGDLA

SEQ ID NO: 16 - protein, 8 aa, Artificial Sequence
  Cyclic peptide
  MISC_FEATURE (6)..(6): Two hexyloxycarbonyl (Hoc) moieties
LPPGLRGD

SEQ ID NO: 17 - protein, 9 aa, Artificial Sequence
  Cyclic peptide
LPPFRGDLA

SEQ ID NO: 18 - protein, 8 aa, Artificial Sequence
  Cyclic peptide
LPPGLRGD

SEQ ID NO: 19 - protein, 6 aa, Artificial Sequence
  Cyclic peptide
  MISC_FEATURE (1)..(1): D-amino acid
AAAAAA

SEQ ID NO: 20 - protein, 5 aa, Artificial Sequence
  Cyclic peptide
  MISC_FEATURE (1)..(1): D-amino acid
  MISC_FEATURE (2)..(2): N methylated
FVRGD

SEQ ID NO: 21 - protein, 6 aa, Artificial Sequence
  Cyclic peptide
  MISC_FEATURE (1)..(1): D-amino acid
  MISC_FEATURE (1)..(1): N methylated
  MISC_FEATURE (2)..(2): Hexyloxycarbonyl (Hoc) moiety
  MISC_FEATURE (4)..(4): Methyl ester (OMe) moiety
  MISC_FEATURE (6)..(6): N methylated
VRGDAA

SEQ ID NO: 22 - protein, 6 aa, Artificial sequence
  Cyclic peptide
  MISC_FEATURE (1)..(1): D-amino acid
  MISC_FEATURE (2)..(2): N methylayed
  MISC_FEATURE (3)..(3): Two hexyloxycarbonyl (Hoc) moieties
AAAAAA

SEQ ID NO: 23 - protein, 5 aa, Artificial sequence
  Cyclic peptide
  MISC_FEATURE (1)..(1): D-amino acid
  MISC_FEATURE (2)..(2): N methylated
  MISC_FEATURE (3)..(3): Two hexyloxycarbonyl (Hoc) moieties
FVRGD

SEQ ID NO: 24 - protein, 9 aa, Artificial sequence
  Peptide
RTDLDSLRT